European Patent Application EP 4 285 729 A2, published December 6, 2023. Title: Cell-associated heterologous food and/or feed enzymes. Applicant: Lallemand Hungary Liquidity Management LLC. Application EP. The sequence listing filed with the application follows.

SEQUENCE LISTING (108 sequences)

SEQ ID NO: 1 - protein, 719 aa, Geobacillus stearothermophilus
MKKKTLSLFVGLMLLIGLLFSGSLPYNPNAAEASSSASVKGDVIYQIIIDRFYDGDTTNNNPAKSYGLYDPTKSKWKMYWGGDLEGVRQKLPYLKQLGVTTIWLSPVLDNLDTLAGTDNTGYHGYWTRDFKQIEEHFGNWTTFDTLVNDAHQNGIKVIVDFVPNHSTPFKANDSTFAEGGALYNNGTYMGNYFDDATKGYFHHNGDISNWDDRYEAQWKNFTDPAGFSLADLSQENGTIAQYLTDAAVQLVAHGADGLRIDAVKHFNSGFSKSLADKLYQKKDIFLVGEWYGDDPGTANHLEKVRYANNSGVNVLDFDLNTVIRNVFGTFTQTMYDLNNMVNQTGNEYKYKENLITFIDNHDMSRFLSVNSNKANLHQALAFILTSRGTPSIYYGTEQYMAGGNDPYNRGMMPAFDTTTTAFKEVSTLAGLRRNNAAIQYGTTTQRWINNDVYIYERKFFNDVVLVAINRNTQSSYSISGLQTALPNGSYADYLSGLLGGNGISVSNGSVASFTLAPGAVSVWQYSTSASAPQIGSVAPNMGIPGNVVTIDGKGFGTTQGTVTFGGVTATVKSWTSNRIEVYVPNMAAGLTDVKVTAGGVSSNLYSYNILSGTQTSVVFTVKSAPPTNLGDKIYLTGNIPELGNWSTDTSGAVNNAQGPLLAPNYPDWFYVFSVPAGKTIQFKFFIKRADGTIQWENGSNHVATTPTGATGNITVTWQN

SEQ ID NO: 2 - protein, 499 aa, Aspergillus oryzae
MMVAWWSLFLYGLQVAAPALAATPADWRSQSIYFLLTDRFARTDGSTTATCNTADRKYCGGTWQGIIDKLDYIQGMGFTAIWITPVTAQLPQTTAYGDAYHGYWQQDIYSLNENYGTADDLKALSSALHERGMYLMVDVVANHMGYDGAGSSVDYSVFKPFSSQDYFHPFCLIQNYEDQTQVEDCWLGDNTVSLPDLDTTKDVVKNEWYDWVGSLVSNYSIDGLRIDTVKHVQKDFWPGYNKAAGVYCIGEVLDGDPAYTCPYQNVMDGVLNYPIYYPLLNAFKSTSGSMDDLYNMINTVKSDCPDSTLLGTFVENHDNPRFASYTNDIALAKNVAAFIILNDGIPIIYAGQEQHYAGGNDPANREATWLSGYPTDSELYKLIASANAIRNYAISKDTGFVTYKNWPIYKDDTTIAMRKGTDGSQIVTILSNKGASGDSYTLSLSGAGYTAGQQLTEVIGCTTVTVGSDGNVPVPMAGGLPRVLYPTEKLAGSKICSSS

SEQ ID NO: 3 - protein, 515 aa, Saccharomycopsis fibuligera
MIRLTVFLTAVFAAVASCVPVELDKRNTGHFQAYSGYTVARSNFTQWIHEQPAVSWYYLLQNIDYPEGQFKSAKPGVVVASPSTSEPDYFYQWTRDTAITFLSLIAEVEDHSFSNTTLAKVVEYYISNTYTLQRVSNPSGNFDSPNHDGLGEPKFNVDDTAYTASWGRPQNDGPALRAYAISRYLNAVAKHNNGKLLLAGQNGIPYSSASDIYWKIIKPDLQHVSTHWSTSGFDLWEENQGTHFFTALVQLKALSYGIPLSKTYNDPGFTSWLEKQKDALNSYINSSGFVNSGKKHIVESPQLSSRGGLDSATYIAALITHDIGDDDTYTPFNVDNSYVLNSLYYLLVDNKNRYKINGNYKAGAAVGRYPEDVYNGVGTSEGNPWQLATAYAGQTFYTLAYNSLKNKKNLVIEKLNYDLYNSFIADLSKIDSSYASKDSLTLTYGSDNYKNVIKSLLQFGDSFLKVLLDHIDDNGQLTEEINRYTGFQAGAVSLTWSSGSLLSANRARNKLIELL

SEQ ID NO: 4 - protein, 551 aa, Pseudomonas saccharophila
MSHILRAAVLAAVLLPFPALADQAGKSPAGVRYHGGDEIILQGFHWNVVREAPNDWYNILRQQASTIAADGFSAIWMPVPWRDFSSWTDGGKSGGGEGYFWHDFNKNGRYGSDAQLRQAAGALGGAGVKVLYDVVPNHMNRGYPDKEINLPAGQGFWRNDCADPGNYPNDCDDGDRFIGGESDLNTGHPQIYGMFRDELANLRSGYGAGGFRFDFVRGYAPERVDSWMSDSADSSFCVGELWKGPSEYPSWDWRNTASWQQIIKDWSDRAKCPVFDFALKERMQNGSVADWKHGLNGNPDPRWREVAVTFVDNHDTGYSPGQNGGQHHWALQDGLIRQAYAYILTSPGTPVVYWSHMYDWGYGDFIRQLIQVRRTAGVRADSAISFHSGYSGLVATVSGSQQTLVVALNSDLANPGQVASGSFSEAVNASNGQVRVWRSGSGDGGGNDGGEGGLVNVNFRCDNGVTQMGDSVYAVGNVSQLGNWSPASAVRLTDTSSYPTWKGSIALPDGQNVEWKCLIRNEADATLVRQWQSGGNNQVQAAAGASTSGSF

SEQ ID NO: 5 - protein, 926 aa, Bacillus naganoensis
DGNTTNIVVHYFRPSGDYTDWNLWMWPENGDGAEYDFNQPTDSYGEVASVDIPGNPSQVGIIVRKGNWDAKDIDSDRYIDLSKGHEIWLVQGNSQIFYSEKDAEAAAQPAVSNAYLDASNQVLVKLSQPFTLGEGSSGFTVHDDTANKDIPVTSVSDANQVTAVLAGTFQHIFGGSDWAPDNHNTLLKKVNSNLYQFSGNLPEGNYQYKVALNDSWNNPSYPSDNINLTVPAGGAHVTFSYIPSTHAVYDTINNPNADLQVDSSGVKTDLVAVTLGENPDVSHTLSIQTEDYQAGQVIPRKVLDSSQYYYSGDDLGNTYTKNATTFKVWAPTSTQVNVLLYNSATGAVTKTVPMTASGHGVWEATVNQDLENWYYMYEVTGQGSTRTAVDPYATAIAPNGTRGMIVDLAKTDPAGWESDKHITPKNIEDEVIYEMDVRDFSIDSNSGMKNKGKYLALTEKGTKGPDNVKTGVDSLKQLGITHVQLQPVFAFNSVNENDPTQYNWGYDPRNYNVPEGQYATNANGTTRIKEFKEMVLSLHQDHIGVNMDVVYNHTFATQISDFDKIVPEYYYRTDDAGNYTNGSGTGNEIAAERPMVQKFIIDSLKFWVNEYHVDGFRFDLMALLGKDTMSKAATQLHAIDPGIALYGEPWTGGTSALPADQLLTKGAQKGMGVAVFNDNLRNGLDGSVFDSSAQGFATGATGLTDAIKNGVEGSINDFTASPGETINYVTSHDNYTLWDKIAQSNPNDSEADRIKMDELAQAIVMTSQGIPFMQGGEEMLRTKGGNDNSYNAGDVVNEFDWSRKAQYPDVFNYYSGLIHLRLDHPAFRMTTANEINSHLQFLNSPENTVAYELSDHANKDTWGNIVVIYNPNKTAETINLPSGKWEINATSGKVGESTLGQAEGSVQVPGISMMILHQEVSPSDGK

SEQ ID NO: 6 - protein, 829 aa, Bacillus acidopullulyticus
DSTSTEVIVHYHRFDSNYANWDLWMWPYQPVNGNGAAYEFSGKDDFGVKADVQVPGDDTQVGLIVRTNDWSQKNTSDDLHIDLTKGHEIWIVQGDPNIYYNLSDAQAAATPKVSNAYLDNEKTVLAKLTNPMTLSDGSSGFTVTDKTTGEQIPVTAATNANSASSSEQTDLVQLTLASAPDVSHTIQVGAAGYEAVNLIPRNVLNLPRYYYSGNDLGNVYSNKATAFRVWAPTASDVQLLLYNSETGPVTKQLEMQKSDNGTWKLKVPGNLKNWYYLYQVTVNGKTQTAVDPYVRAISVNATRGMIVDLEDTNPPGWKEDHQQTPANPVDEVIYEVHVRDFSIDANSGMKNKGKYLAFTEHGTKGPDNVKTGIDSLKELGINAVQLQPIEEFNSIDETQPNMYNWGYDPRNYNVPEGAYATTPEGTARITQLKQLIQSIHKDRIAINMDVVYNHTFNVGVSDFDKIVPQYYYRTDSAGNYTNGSGVGNEIATERPMVQKFVLDSVKYWVKEYHIDGFRFDLMALLGKDTMAKISKELHAINPGIVLYGEPWTGGTSGLSSDQLVTKGQQKGLGIGVFNDNIRNGLDGNVFDKSAQGFATGDPNQVNVIKNRVMGSISDFTSAPSETINYVTSHDNMTLWDKISASNPNDTQADRIKMDELAQAVVFTSQGVPFMQGGEEMLRTKGGNDNSYNAGDSVNQFDWSRKAQFENVFDYYSWLIHLRDNHPAFRMTTADQIKQNLTFLDSPTNTVAFELKNHANHDKWKNIIVMYNPNKTAQTLTLPSGNWTIVGLGNQVGEKSLGHVNGTVEVPALSTIILHQGTSEDVIDQN

SEQ ID NO: 7 - protein, 776 aa, Pseudomonas amyloderamosa
MKCPKILAALLGCAVLAGVPAMPAHAAINSMSLGASYDAQQANITFRVYSSQATRIVLYLYSAGYGVQESATYTLSPAGSGVWAVTVPVSSIKAAGITGAVYYGYRAWGPNWPYASNWGKGSQAGFVSDVDANGDRFNPNKLLLDPYAQEVSQDPLNPSNQNGNVFASGASYRTTDSGIYAPKGVVLVPSTQSTGTKPTRAQKDDVIYEVHVRGFTEQDTSIPAQYRGTYYGAGLKASYLASLGVTAVEFLPVQETQNDANDVVPNSDANQNYWGYMTENYFSPDRRYAYNKAAGGPTAEFQAMVQAFHNAGIKVYMDVVYNHTAEGGTWTSSDPTTATIYSWRGLDNATYYELTSGNQYFYDNTGIGANFNTYNTVAQNLIVDSLAYWANTMGVDGFRFDLASVLGNSCLNGAYTASAPNCPNGGYNFDAADSNVAINRILREFTVRPAAGGSGLDLFAEPWAIGGNSYQLGGFPQGWSEWNGLFRDSLRQAQNELGSMTIYVTQDANDFSGSSNLFQSSGRSPWNSINFIDVHDGMTLKDVYSCNGANNSQAWPYGPSDGGTSTNYSWDQGMSAGTGAAVDQRRAARTGMAFEMLSAGTPLMQGGDEYLRTLQCNNNAYNLDSSANWLTYSWTTDQSNFYTFAQRLIAFRKAHPALRPSSWYSGSQLTWYQPSGAVADSNYWNNTSNYAIAYAINGPSLGDSNSIYVAYNGWSSSVTFTLPAPPSGTQWYRVTDTCDWNDGASTFVAPGSETLIGGAGTTYGQCGQSLLLLISK

SEQ ID NO: 8 - protein, 500 aa, Thermus thermophilus
MELPRAFGLLLHPTSLPGPYGVGVLGQEARDFLRFLKEAGGRYWQVLPLGPTGYGDSPYQSFSAFAGNPYLIDLRPLAERGYVRLEDPGFPQGRVDYGLLYAWKWPALKEAFRGFKEKASPEEREAFAAFREREAWWLEDYALFMALKGAHGGLPWNRWPLPLRKREEKALREAKSALAEEVAFHAFTQWLFFRQWGALKAEAEALGIRIIGDMPIFVAEDSAEVWAHPEWFHLDEEGRPTVVAGVPPDYFSETGQRWGNPLYRWDVLEREGFSFWIRRLEKALELFHLVRIDHFRGFEAYWEIPASCPTAVEGRWVKAPGEKLFQKIQEVFGEVPVLAEDLGVITPEVEALRDRFGLPGMKVLQFAFDDGMENPFLPHNYPAHGRVVVYTGTHDNDTTLGWYRTATPHEKAFMARYLADWGITFREEEEVPWALMHLGMKSVARLAVYPVQDVLALGSEARMNYPGRPSGNWAWRLLPGELSPEHGARLRAMAEATERL

SEQ ID NO: 9 - DNA, 1641 bp, synthetic construct
  misc_feature 1..1641: note = Flo1 tether
  source 1..1641: mol_type = other DNA
  CDS 1..1641
aaggacaatagctcgacgattgaaggtagatacccatacgacgttccagactacgctctgcaggctagtggtggtggtggttctggtggtggtggttctggtggtggtggttctgctagcatcagaactccaaccagtgaaggtttggttacaaccaccactgaaccatggactggtacttttacttcgacttccactgaaatgtctactgtcactggaaccaatggcttgccaactgatgaaactgtcattgttgtcaaaactccaactactgccatctcatccagtttgtcatcatcatcttcaggacaaatcaccagctctatcacgtcttcgcgtccaattattaccccattctatcctagcaatggaacttctgtgatttcttcctcagtaatttcttcctcagtcacttcttctctattcacttcttctccagtcatttcttcctcagtcatttcttcttctacaacaacctccacttctatattttctgaatcatctaaatcatccgtcattccaaccagtagttccacctctggttcttctgagagcgaaacgagttcagctggttctgtctcttcttcctcttttatctcttctgaatcatcaaaatctcctacatattcttcttcatcattaccacttgttaccagtgcgacaacaagccaggaaactgcttcttcattaccacctgctaccactacaaaaacgagcgaacaaaccactttggttaccgtgacatcctgcgagtctcatgtgtgcactgaatccatctcccctgcgattgtttccacagctactgttactgttagcggcgtcacaacagagtataccacatggtgccctatttctactacagagacaacaaagcaaaccaaagggacaacagagcaaaccacagaaacaacaaaacaaaccacggtagttacaatttcttcttgtgaatctgacgtatgctctaagactgcttctccagccattgtatctacaagcactgctactattaacggcgttactacagaatacacaacatggtgtcctatttccaccacagaatcgaggcaacaaacaacgctagttactgttacttcctgcgaatctggtgtgtgttccgaaactgcttcacctgccattgtttcgacggccacggctactgtgaatgatgttgttacggtctatcctacatggaggccacagactgcgaatgaagagtctgtcagctctaaaatgaacagtgctaccggtgagacaacaaccaatactttagctgctgaaacgactaccaatactgtagctgctgagacgattaccaatactggagctgctgagacgaaaacagtagtcacctcttcgctttcaagatctaatcacgctgaaacacagacggcttccgcgaccgatgtgattggtcacagcagtagtgttgtttctgtatccgaaactggcaacaccaagagtctaacaagttccgggttgagtactatgtcgcaacagcctcgtagcacaccagcaagcagcatggtaggatatagtacagcttctttagaaatttcaacgtatgctggcagtgccaacagcttactggccggtagtggtttaagtgtcttcattgcgtccttattgctggcaattatttaa

SEQ ID NO: 10 - protein, 546 aa, synthetic construct
  REGION 1..546: note = Synthetic Construct
KDNSSTIEGRYPYDVPDYALQASGGGGSGGGGSGGGGSASIRTPTSEGLVTTTTEPWTGTFTSTSTEMSTVTGTNGLPTDETVIVVKTPTTAISSSLSSSSSGQITSSITSSRPIITPFYPSNGTSVISSSVISSSVTSSLFTSSPVISSSVISSSTTTSTSIFSESSKSSVIPTSSSTSGSSESETSSAGSVSSSSFISSESSKSPTYSSSSLPLVTSATTSQETASSLPPATTTKTSEQTTLVTVTSCESHVCTESISPAIVSTATVTVSGVTTEYTTWCPISTTETTKQTKGTTEQTTETTKQTTVVTISSCESDVCSKTASPAIVSTSTATINGVTTEYTTWCPISTTESRQQTTLVTVTSCESGVCSETASPAIVSTATATVNDVVTVYPTWRPQTANEESVSSKMNSATGETTTNTLAAETTTNTVAAETITNTGAAETKTVVTSSLSRSNHAETQTASATDVIGHSSSVVSVSETGNTKSLTSSGLSTMSQQPRSTPASSMVGYSTASLEISTYAGSANSLLAGSGLSVFIASLLLAII

SEQ ID NO: 11 - DNA, 807 bp, synthetic construct
  misc_feature 1..807: note = Sed1 tether
  source 1..807: mol_type = other DNA
  CDS 1..807
aaggacaatagctcgacgattgaaggtagatacccatacgacgttccagactacgctctgcaggctagtggtggtggtggttctggtggtggtggttctggtggtggtggttctgctagcgctcttccaactaacggtacttctactgaagctccaactgatactactactgaagctccaaccaccggtcttccaaccaacggtaccacttcagctttcccaccaactacatctttgccaccaagcaacactaccaccactcctccttacaacccatctactgactacaccactgactacactgtagtcactgaatatactacttactgtccagaaccaaccactttcaccacaaacggtaagacttacaccgtcactgaaccaaccacattgactatcactgactgtccatgcaccattgaaaagccaacaaccacatcaaccaccgaatacactgtagtcactgagtacactacttactgtccagaaccaaccactttcaccacaaacggtaagacttacaccgtcactgaaccaaccactttgactatcactgactgtccatgtactattgaaaagagcgaagcccctgagtcttctgtcccagttaccgaatctaagggcactaccaccaaagaaacaggtgttactaccaaacaaaccacagccaacccaagtctaaccgtctccacagtcgtcccagtttcatcctctgcttcttctcattccgttgtcatcaacagtaacggtgctaacgtcgtcgttccaggtgctttaggtttggctggtgttgctatgttattctaa

SEQ ID NO: 12 - protein, 268 aa, synthetic construct
  REGION 1..268: note = Synthetic Construct
KDNSSTIEGRYPYDVPDYALQASGGGGSGGGGSGGGGSASALPTNGTSTEAPTDTTTEAPTTGLPTNGTTSAFPPTTSLPPSNTTTTPPYNPSTDYTTDYTVVTEYTTYCPEPTTFTTNGKTYTVTEPTTLTITDCPCTIEKPTTTSTTEYTVVTEYTTYCPEPTTFTTNGKTYTVTEPTTLTITDCPCTIEKSEAPESSVPVTESKGTTTKETGVTTKQTTANPSLTVSTVVPVSSSASSHSVVINSNGANVVVPGALGLAGVAMLF

SEQ ID NO: 13 - DNA, 759 bp, synthetic construct
  misc_feature 1..759: note = Tir1 tether
  source 1..759: mol_type = other DNA
  CDS 1..759
aaggacaatagctcgacgattgaaggtagatacccatacgacgttccagactacgctctgcaggctagtggtggtggtggttctggtggtggtggttctggtggtggtggttctgctagcagcttagcttctgattcttcctctggattttccttaagcagtatgccagctggtgttttggatatcggtatggctttagcttccgccactgacgactcctacactactttgtactctgaggttgactttgctggtgttagcaagatgttgaccatggttccatggtactcctctagattggaaccagctttgaagtctttgaatggtgatgcttcttcttctgctgccccaagctcttctgctgctccaacttcttctgctgccccaagctcatctgctgccccaacttcttctgctgcctcaagctcttctgaagctaagtcttcttctgctgccccaagctcttctgaagctaagtcttcttctgctgccccaagctcttctgaagctaagtcttcttctgctgccccaagctcttctgaagctaagtcttcttctgctgctccaagctccactgaagctaagataacttctgctgctccaagctccactggtgccaagacctctgccatctctcaaattaccgatggtcaaatccaagctaccaaggctgtttctgagcaaactgaaaacggtgctgctaaggcctttgttggtatgggtgctggtgttgtcgcagctgccgctatgttgttataa

SEQ ID NO: 14 - protein, 252 aa, synthetic construct
  REGION 1..252: note = Synthetic Construct
KDNSSTIEGRYPYDVPDYALQASGGGGSGGGGSGGGGSASSLASDSSSGFSLSSMPAGVLDIGMALASATDDSYTTLYSEVDFAGVSKMLTMVPWYSSRLEPALKSLNGDASSSAAPSSSAAPTSSAAPSSSAAPTSSAASSSSEAKSSSAAPSSSEAKSSSAAPSSSEAKSSSAAPSSSEAKSSSAAPSSTEAKITSAAPSSTGAKTSAISQITDGQIQATKAVSEQTENGAAKAFVGMGAGVVAAAAMLL

SEQ ID NO: 15 - DNA, 450 bp, synthetic construct
  misc_feature 1..450: note = Cwp2 tether
  source 1..450: mol_type = other DNA
  CDS 1..450
aaggacaatagctcgacgattgaaggtagatacccatacgacgttccagactacgctctgcaggctagtggtggtggtggttctggtggtggtggttctggtggtggtggttctgctagcggatccggtggcggtggatctggaggaggcggttcttggtctcacccacaatttgaaaagggtggagaaaacttgtactttcaaggcggtggtggaggttctggcggaggtggctccggctcagctatctctcaaatcaccgacggtcaaatccaagccactaccacagctaccactgaagctacaactaccgctgctccttcatctactgttgaaactgtttctccatcttccaccgaaaccatctctcaacaaaccgaaaacggtgctgctaaggctgctgttggtatgggtgctggtgctttggctgctgctgctatgttgttgtaa

SEQ ID NO: 16 - protein, 149 aa, synthetic construct
  REGION 1..149: note = Synthetic Construct
KDNSSTIEGRYPYDVPDYALQASGGGGSGGGGSGGGGSASGSGGGGSGGGGSWSHPQFEKGGENLYFQGGGGGSGGGGSGSAISQITDGQIQATTTATTEATTTAAPSSTVETVSPSSTETISQQTENGAAKAAVGMGAGALAAAAMLL

SEQ ID NO: 17 - DNA, 468 bp, synthetic construct
  misc_feature 1..468: note = Ccw12 tether
  source 1..468: mol_type = other DNA
  CDS 1..468
aaggacaatagctcgacgattgaaggtagatacccatacgacgttccagactacgctctgcaggctagtggtggtggtggttctggtggtggtggttctggtggtggtggttctgctagcgctgctaacgttaccactgctactgtcagccaagaatctaccactttggtcaccatcacttcttgtgaagaccacgtctgttctgaaactgtctccccagctttggtttccaccgctaccgtcaccgtcgatgacgttatcactcaatacaccacctggtgcccattgaccactgaagccccaaagaacggtacttctactgctgctccagttacctctactgaagctccaaagaacaccacctctgctgctccaactcactctgtcacctcttacactggtgctgctgctaaggctttgccagctgctggtgctttgttggctggtgccgctgctttgttgttgtaa

SEQ ID NO: 18 - protein, 155 aa, synthetic construct
  REGION 1..155: note = Synthetic Construct
KDNSSTIEGRYPYDVPDYALQASGGGGSGGGGSGGGGSASAANVTTATVSQESTTLVTITSCEDHVCSETVSPALVSTATVTVDDVITQYTTWCPLTTEAPKNGTSTAAPVTSTEAPKNTTSAAPTHSVTSYTGAAAKALPAAGALLAGAAALLL

SEQ ID NO: 19 - DNA, 510 bp, synthetic construct
  misc_feature 1..510: note = Spi1 tether
  source 1..510: mol_type = other DNA
  CDS 1..510
aaggacaatagctcgacgattgaaggtagatacccatacgacgttccagactacgctctgcaggctagtggtggtggtggttctggtggtggtggttctggtggtggtggttctgctagcttggtatctaattctagttcctctgtaatcgtggtaccatcaagcgatgctactattgccggtaacgatacagccacgccagcaccagagccatcatccgccgctccaatattctacaactcgactgctactgcaacacagtacgaagttgtcagtgaattcactacttactgcccagaaccaacgactttcgtaacgaatggcgctacattcactgttactgccccaactacgttaacaattaccaactgtccttgcactatcgagaagcctacttcagaaacatcggtttcttctacacatgatgtggagacaaattctaatgctgctaacgcaagagcaatcccaggagccctaggtttggctggtgcagttatgatgcttttatga

SEQ ID NO: 20 - protein, 169 aa, synthetic construct
  REGION 1..169: note = Synthetic Construct
KDNSSTIEGRYPYDVPDYALQASGGGGSGGGGSGGGGSASLVSNSSSSVIVVPSSDATIAGNDTATPAPEPSSAAPIFYNSTATATQYEVVSEFTTYCPEPTTFVTNGATFTVTAPTTLTITNCPCTIEKPTSETSVSSTHDVETNSNAANARAIPGALGLAGAVMMLL

SEQ ID NO: 21 - DNA, 1398 bp, synthetic construct
  misc_feature 1..1398: note = Pst1 tether
  source 1..1398: mol_type = other DNA
  CDS 1..1398
aaggacaatagctcgacgattgaaggtagatacccatacgacgttccagactacgctctgcaggctagtggtggtggtggttctggtggtggtggttctggtggtggtggttctgctagcgctacttcctcttcttccagcataccctcttcctgtaccataagctcacatgccacggccacagctcagagtgacttagataaatatagccgctgtgatacgttagtcgggaacttaactattggtggtggtttgaagactggtgctttggctaatgttaaagaaatcaacgggtctctaactatatttaacgctacaaatctaacctcattcgctgctgattccttggagtccatcacagattctttgaacctacagagtttgacaatcttgacttctgcttcatttgggtctttacagagcgttgatagtataaaactgattactctacccgccatctccagttttacttcaaatatcaaatctgctaacaacatttatatttccgacacttcgttacaatctgtcgatggattctcagccttgaaaaaagttaacgtgttcaacgtcaataacaataagaaattaacctcgatcaaatctccagttgaaacagtcagcgattctttacaattttcgttcaacggtaaccagactaaaatcaccttcgatgacttggtttgggcaaacaatatcagtttgaccgatgtccactctgtttccttcgctaacttgcaaaagattaactcttcattgggtttcatcaacaactccatctcaagtttgaatttcactaagctaaacaccattggccaaaccttcagtatcgtttccaatgactacttgaagaacttgtcgttctctaatttgtcaaccataggtggtgctcttgtcgttgctaacaacactggtttacaaaaaattggtggtctcgacaacctaacaaccattggcggtactttggaagttgttggtaacttcacctccttgaacctagactctttgaagtctgtcaagggtggcgcagatgtcgaatcaaagtcaagcaatttctcctgtaatgctttgaaagctttgcaaaagaaagggggtatcaagggtgaatcttttgtctgcaaaaatggtgcatcatccacatctgttaaactatcgtccacttccaaatctcaatcaagccaaactactgccaaggtttccaagtcatcttctaaggccgaggaaaagaagttcacttctggcgatatcaaggctgctgcttctgcctctagtgtttctagttctggcgcttccagctctagctctaagagttccaaaggcaatgccgctatcatggcaccaattggccaaacaacccctttggtcggtcttttgacggcaatcatcatgtctataatgtaa

SEQ ID NO: 22 - protein, 465 aa, synthetic construct
  REGION 1..465: note = Synthetic Construct
KDNSSTIEGRYPYDVPDYALQASGGGGSGGGGSGGGGSASATSSSSSIPSSCTISSHATATAQSDLDKYSRCDTLVGNLTIGGGLKTGALANVKEINGSLTIFNATNLTSFAADSLESITDSLNLQSLTILTSASFGSLQSVDSIKLITLPAISSFTSNIKSANNIYISDTSLQSVDGFSALKKVNVFNVNNNKKLTSIKSPVETVSDSLQFSFNGNQTKITFDDLVWANNISLTDVHSVSFANLQKINSSLGFINNSISSLNFTKLNTIGQTFSIVSNDYLKNLSFSNLSTIGGALVVANNTGLQKIGGLDNLTTIGGTLEVVGNFTSLNLDSLKSVKGGADVESKSSNFSCNALKALQKKGGIKGESFVCKNGASSTSVKLSSTSKSQSSQTTAKVSKSSSKAEEKKFTSGDIKAAASASSVSSSGASSSSSKSSKGNAAIMAPIGQTTPLVGLLTAIIMSIM

SEQ ID NO: 23 - DNA, 330 bp, synthetic construct
  misc_feature 1..330: note = Aga1/2 tether
  source 1..330: mol_type = other DNA
  CDS 1..330
aaggacaatagctcgacgattgaaggtagatacccatacgacgttccagactacgctctgcaggctagtggtggtggtggttctggtggtggtggttctggtggtggtggttctgctagccaggaactgacaactatatgcgagcaaatcccctcaccaactttagaatcgacgccgtactctttgtcaacgactactattttggccaacgggaaggcaatgcaaggagtttttgaatattacaaatcagtaacgtttgtcagtaattgcggttctcacccctcaacaactagcaaaggcagccccataaacacacagtatgttttttaa

SEQ ID NO: 24 - protein, 109 aa, synthetic construct
  REGION 1..109: note = Synthetic Construct
KDNSSTIEGRYPYDVPDYALQASGGGGSGGGGSGGGGSASQELTTICEQIPSPTLESTPYSLSTTTILANGKAMQGVFEYYKSVTFVSNCGSHPSTTSKGSPINTQYVF

SEQ ID NO: 25 - DNA, 381 bp, synthetic construct
  misc_feature 1..381: note = Aga1/2 tether
  source 1..381: mol_type = other DNA
  CDS 1..381
atgcagttacttcgctgtttttcaatattttctgttattgcttcagttttagcacaggagctgacaactatatgcgagcaaatcccctcaccaactttagaatcgacgccgtactctttgtcaacgactactattttggccaacgggaaggcaatgcaaggagtttttgaatattacaaatcagtaacgtttgtcagtaattgcgattctcacccctcaacaactagcaaagacagccccataaacacacagtatgtttttaaggacaatagctcgacgattgaaggtagatacccatacgacgttccagactacgctctgcaggctagtggtggtggtggttctggtggtggtggttctggtggtggtggttctgctagc

SEQ ID NO: 26 - protein, 127 aa, synthetic construct
  REGION 1..127: note = Synthetic Construct
MQLLRCFSIFSVIASVLAQELTTICEQIPSPTLESTPYSLSTTTILANGKAMQGVFEYYKSVTFVSNCDSHPSTTSKDSPINTQYVFKDNSSTIEGRYPYDVPDYALQASGGGGSGGGGSGGGGSAS

SEQ ID NO: 27 - DNA, 750 bp, synthetic construct
  misc_feature 1..750: note = Promoter of tdh1 gene
  source 1..750: mol_type = other DNA
agaaacgaatgtatatgctcatttacactctatatcaccatatggaggataagttgggctgagcttctgatccaatttattctatccattagttgctgatatgtcccaccagccaacacttgatagtatctactcgccattcacttccagcagcgccagtagggttgttgagcttagtaaaaatgtgcgcaccacaagcctacatgactccacgtcacatgaaaccacaccgtggggccttgttacgctaggaataggatatgcgacgaagacgcttctgcttagtaaccacaccacattttcaaggggtcgatctgcttgcttcctttactgtcacgagcggcccataatcgcgctttttttttaaaatgcgcgagacagcaaacaggaagctcgggtttcaaccttcggagtggtcgcagatctggagactggatccttacaatacagtaaggcaagccaccatctgcttcttaggtgcatgcgacggtatccacgtgcagaacaacatagtctgaagaagggggggaggagcatgttcattctctgtagcactaagagcttggtgataatgaccaaaactggagtctcgaaatcatataaatagacaatatattttcacacaatgtgatttgtagtacagttctactctctctcttgcataaataagaaattcatcaagaacttggtttgatatttcaccaacacacacaaaaaacagtacttcactaaatttacacacaaaacaaa

SEQ ID NO: 28 - DNA, 750 bp, synthetic construct
  misc_feature 1..750: note = Promotoer of hor7 gene
  source 1..750: mol_type = other DNA
acctccatgaaatttttttttttctttcgattagcacgcacacacatcacatagactgcgtcataaaaatacactacggaaaaaccataaagagcaaagcgatacctacttggaaggaaaaggagcacgcttgtaagggggatgggggctaagaagtcattcactttcttttcccttcgcggtccggacccgggacccctcctctccccgcacaatttcttcctttcatatcttccttttattcctatcccgttgaagcaaccgcactatgactaaatggtgctggacatctccatggctgtgacttgtgtgtatctcacagtggtaacggcaccgtggctcggaaacggttccttcgtgacaattctagaacaggggctacagtctcgataatagaataataagcgcatttttgttagcgccgccgcggcgcccgtttcccaatagggaggcgcagtttatcggcggagctttacttcttcctatttgggtaagcccctttctgttttcggccagtggttgctgcaggctgcgccggagaacatagtgataagggatgtaactttcgatgagagaattagcaagcggaaaaaaaactatggctagctgggagttgtttttcaatcatataaaagggagaaattgttgctcactatgtgacagtttctgggacgtcttaacttttattgcagaggactatcaaatcatacagatattgtcaaaaaaaaaaaaaaagactaataataaaaa

SEQ ID NO: 29 - DNA, 750 bp, synthetic construct
  misc_feature 1..750: note = Promoter of hsp150 gene
  source 1..750: mol_type = other DNA
tgtaaaaacaagcaaaaaaaaaccaagaaggaacaaatgcaccaaactgttgatctattctgcaaaaaaagtatggtaaattttttccattatcctggccgctaatccatatggaggtgaacttagaacttgcacaaggatgcgatgaatgataggctttgtgctataattaatgcaggcaggtccgccatgtccaacacgttgctggccgcaaaacgagtcaatctcactgctttgccacgctcatttctccccccttctgcccaattaggcgaccctcacaatgcacatacacatttcccacctctattggaaggggccgtaaatggtaattcttgggagttattcatattaagtgatcttactatttcctatttcggaaattattaaagacaaaaaagctcatttatggctttccgtctgtagtgataagtcgccaactcagcctaatttttcatttctttaccagatcaggaaaactaatagtacaaatgagttttttctcaagcggaacaccacattttgagctaaatttagattttggtcaaaataagaaagatcctaaaaaaggaatggttggtgaaaaatttattagcttgaatggtaggaatcctcgagatataaaaggaacacttgaagtctaacgacaatcaatttcgattatgtccttccttttacctcaaagctcaaaaaaacatcaataagaaactcatattccttttctaaccctagtacaataataataatata

SEQ ID NO: 30 - DNA, 450 bp, synthetic construct
  misc_feature 1..450: note = Promoter of hxt7 gene
  source 1..450: mol_type = other DNA
ccagaaaggcaacgcaaaattttttttccagggaataaactttttatgacccactacttctcgtaggaacaatttcgggcccctgcgtgttcttctgaggttcatcttttacatttgcttctgctggataattttcagaggcaacaaggaaaaattagatggcaaaaagtcgtctttcaaggaaaaatccccaccatctttcgagatcccctgtaacttattggcaactgaaagaatgaaaaggaggaaaatacaaaatatactagaactgaaaaaaaaaaagtataaatagagacgatatatgccaatacttcacaatgttcgaatctattcttcatttgcagctattgtaaaataataaaacatcaagaacaaacaagctcaacttgtcttttctaagaacaaagaataaacacaaaaacaaaaagtttttttaattttaatcaaaaa

SEQ ID NO: 31 - DNA, 1000 bp, synthetic construct
  misc_feature 1..1000: note = Promoter of gpm1 gene
  source 1..1000: mol_type = other DNA
tgtggtagaattcaaaagactatgtgatgccataggcaagaagggagactctcactccgagatgggcagcttgatcgcccaggaattgaattgtattgtggtggagaaaggtcagtcagataagatattctcacccgatagtgaaaaagacatgttgacgaacagcgaagagggcagcaacaagagggtaggaggccaaggtgatactttgacaggagctatatcatgcatgcttgcatttagtcgtgcaatgtatgactttaagatttgtgagcaggaagaaaagggagaatcttctaacgataaacccttgaaaaactgggtagactacgctatgttgagttgctacgcaggctgcacaattacacgagaatgctcccgcctaggatttaaggctaagggacgtgcaatgcagacgacagatctaaatgaccgtgtcggtgaagtgttcgccaaacttttcggttaacacatgcagtgatgcacgcgcgatggtgctaagttacatatatatatatatatatatatatatatatatatagccatagtgatgtctaagtaacctttatggtatatttcttaatgtggaaagatactagcgcgcgcacccacacacaagcttcgtcttttcttgaagaaaagaggaagctcgctaaatgggattccactttccgttccctgccagctgatggaaaaaggttagtggaacgatgaagaataaaaagagagatccactgaggtgaaatttcagctgacagcgagtttcatgatcgtgatgaacaatggtaacgagttgtggctgttgccagggagggtggttctcaacttttaatgtatggccaaatcgctacttgggtttgttatataacaaagaagaaataatgaactgattctcttcctccttcttgtcctttcttaattctgttgtaattaccttcctttgtaattttttttgtaattattcttcttaataatccaaacaaacacacatattacaata

SEQ ID NO: 32 - DNA, 750 bp, synthetic construct
  misc_feature 1..750: note = Promoter of pgk1 gene
  source 1..750: mol_type = other DNA
acgcacagatattataacatctgcacaataggcatttgcaagaattactcgtgagtaaggaaagagtgaggaactatcgcatacctgcatttaaagatgccgatttgggcgcgaatcctttattttggcttcaccctcatactattatcagggccagaaaaaggaagtgtttccctccttcttgaattgatgttaccctcataaagcacgtggcctcttatcgagaaagaaattaccgtcgctcgtgatttgtttgcaaaaagaacaaaactgaaaaaacccagacacgctcgacttcctgtcttcctattgattgcagcttccaatttcgtcacacaacaaggtcctagcgacggctcacaggttttgtaacaagcaatcgaaggttctggaatggcgggaaagggtttagtaccacatgctatgatgcccactgtgatctccagagcaaagttcgttcgatcgtactgttactctctctctttcaaacagaattgtccgaatcgtgtgacaacaacagcctgttctcacacactcttttcttctaaccaagggggtggtttagtttagtagaacctcgtgaaacttacatttacatatatataaacttgcataaattggtcaatgcaagaaatacatatttggtcttttctaattcgtagtttttcaagttcttagatgctttctttttctcttttttacagatcatcaaggaagtaattatctactttttacaacaaatataaaaca

SEQ ID NO: 33 - DNA, 1020 bp, synthetic construct
  misc_feature 1..1020: note = Promoter of stl1 gene
  source 1..1020: mol_type = other DNA
tggtctcgcgtgtgaatcagcaatgattctgaaatactccttttacaacctttgcaaagataatgtcattcagtctgatattacgagcgacctggaagcactaatccatattcttcattcaacttactccattttccttggcaaacaatgccccacaatcatatacgtcataactataagggatatgtctggaatgcggccaagatagaattaaagggctgcagaacaccactactgatactcattgccaaggctaggaggcaccatccgtttcattttctttgaggtaagccaatcatgaaatagtatacacatccataacggacgtacggacgaaataagtgccgttgtcccactattccaccgcatttggcccatttggctcactttgactcaacttgcgtcattttaactgatatgaagggtccgactttgtcctttttcggccaccgcataccccacggcgacgcctccgctacctgcatttgagtagcatctccgtttcgcggggtattcggcgctacgtcgcctgttcgagcggctctgttcgttgcatgaaactaaaataagcggaaagtgtccagccatccactacgtcagaaagaaataatggttgtacactgtttctcggctatataccgtttttggttggttaatcctcgccaggtgcagctattgcgcttggctgcttcgcgatagtagtaatctgagaaagtgcagatcccggtaagggaaacacttttggttcacctttgatagggctttcattggggcattcgtaacaaaaaggaagtagatagagaaattgagaaagcttaagtgagatgttttagcttcaattttgtccccttcaacgctgcttggccttagagggtcagaattgcagttcaggagtagtcacactcatagtatataaacaagccctttattgattttgaataattattttgtatacgtgttctagcatacaagttagaataaataaaaaatagaaaaatagaacatagaaagttttagacc

SEQ ID NO: 34 - DNA, 500 bp, synthetic construct
  misc_feature 1..500: note = Terminator of dit1 gene
  source 1..500: mol_type = other DNA
taaagtaagagcgctacattggtctacctttttgttcttttacttaaacattagttagttcgttttctttttctcatttttttatgtttcccctcaaaagttctgattttataatattttatttcacacaattccaattaacagagggggaatagattctttagcttagaaaattagtgatcaatatatatttgcctttcttttcatcttttcagtgatattaatggtttcgagacactgcaatggccctagttgtctaagaggatagatgttactgtcaaagatgatattttgaatttcaattgacgtaattaatgatactattaataatacagagcgtatatgaagtattgcaaataacatgcacagttcttttgggatgagaatgagaatgagaggcgaaggcgggcgttcagaaaagcgttgcggagtaacaagtgattaaatagcacccaaataatcttctttgatactaccgattgcgtgaatagaactcactt

SEQ ID NO: 35 - DNA, 500 bp, synthetic construct
  misc_feature 1..500: note = Terminator of idp1 gene
  source 1..500: mol_type = other DNA
tcgaatttacgtagcccaatctaccactttttttttcattttttaaagtgttatacttagttatgctctaggataatgaactacttttttttttttttactgttatcataaatatatataccttattgatgtttgcaaccgtcggttaattccttatcaaggttccccaagttcggatcattaccatcaatttccaacatcttcatgagttcttcttcttcattaccgtgttttagggggctgttcgcacttctaatagggctatcaccaagctgttctaattcgtccaaaagttcagtaacacgatctttatgcttcagttcgtcataatctttcaattcataaatatttacaatttcgtctacgatattaaattgcctcttgtaggtgcctatcttttccttatgctcttcattttcaccgttttcttgaaaccaaacaccgaactcactacgcatttctttcataggctcatataatacttcttttgacgtcatttg

SEQ ID NO: 36 - DNA, 401 bp, synthetic construct
  misc_feature 1..401: note = Terminator of gpm1 gene
  source 1..401: mol_type = other DNA
gtctgaagaatgaatgatttgatgatttctttttccctccatttttcttactgaatatatcaatgatatagacttgtatagtttattatttcaaattaagtagctatatatagtcaagataacgtttgtttgacacgattacattattcgtcgacatcttttttcagcctgtcgtggtagcaatttgaggagtattattaattgaataggttcattttgcgctcgcataaacagttttcgtcagggacagtatgttggaatgagtggtaattaatggtgacatgacatgttatagcaataaccttgatgtttacatcgtagtttaatgtacaccccgcgaattcgttcaagtaggagtgcaccaattgcaaagggaaaagctgaatgggcagttcgaatag

SEQ ID NO: 37 - DNA, 500 bp, synthetic construct
  misc_feature 1..500: note = Terminator of pma1 gene
  source 1..500: mol_type = other DNA
tcctgttgaagtagcatttaatcataatttttgtcacattttaatcaacttgatttttctggtttaatttttctaattttaattttaatttttttatcaatgggaactgatacactaaaaagaattaggagccaacaagaataagccgcttatttcctactagagtttgcttaaaatttcatctcgaattgtcattctaatattttatccacacacacaccttaaaatttttagattaaatggcatcaactcttagcttcacacacacacacacaccgaagctggttgttttatttgatttgatataattggtttctctggatggtactttttctttcttggttatttcctattttaaaatatgaaacgcacacaagtcataattattctaatagagcacaattcacaacacgcacatttcaactttaatatttttttagaaacactttatttagtctaattcttaatttttaatatatataatgcacacacactaattt

SEQ ID NO: 38 - DNA, 500 bp, synthetic construct
  misc_feature 1..500: note = Terminator of tdh3 gene
  source 1..500: mol_type = other DNA
gtgaatttactttaaatcttgcatttaaataaattttctttttatagctttatgacttagtttcaatttatatactattttaatgacattttcgattcattgattgaaagctttgtgttttttcttgatgcggtattgcattgttcttgtctttttcgccacatgtaatatctgtaatagatatctgatacattgtggatgctgagtgaaattttagttaataatggaggcgctcttaataattttggggatattggcttttttttttaaagtttacaaatgaattttttccgccaggataacgattctgaagttactcttagcgttcctatcggtacagccatcaaatcatgcctataaatcatgcctatatttgcgtgcagtcagtatcatctacatgaaaaaaactcccgcaatttcttatagaatacgttgaaaattaaatgtacgcgccaagataagataacataaatctagatgcagtaatatacacagattcc

SEQ ID NO: 39 - DNA, 500 bp, synthetic construct
  misc_feature 1..500: note = Terminator of hxt2 gene
  source 1..500: mol_type = other DNA
gagattatacttaaactagcactgatttttttaaggctaatggctactaatactttaatagatgatcttcatacttttttatttaacgatttttaatgatgtttttatttgtaccactcatttatctagatttttttaatactgatcaaatcttacggactcgacgttaaaaagttcctacatacgtctggtacttgaaacgctgcttcgaggtattgacactataagaatacgatccaaatacttacaccgcatgtaaaaatatgccgacaatatgaatacttgttgatgaatgatatttgattttaatccggcaatttacctcctttatataatccaataattgttgataattagtggttaggttgcagtactaataagaattaagacaaatattcttctactatataaaaggtgcaaacaaaacacacgccgatcggccatactaaacaagaccaacataataatggtggaaccatttactgtattttcaatgtaac

SEQ ID NO: 40 - DNA, 500 bp, synthetic construct
  misc_feature 1..500: note = Terminator of ira2 gene
  source 1..500: mol_type = other DNA
aggtgttacataaactaatgaaagaaatatcaatatctatctgtaagcatgaatgtacatatctcatgttagggttttcttatcgctaatttttcgcaatttgttacgtgggttgcttttatacagctacaatttttatatattctatcatgtaatgaatggctcagtaaattcaagcgccacatagactaatgtacataccaatgcatttaattgtaagaatgaaaggggccattcatctaccgtcttagttgaaagtgtttctgtgaattttttcaaattccgttttttcctttttatataatagcatggtggcgcgagcatcttcgactgaagaatgctcaccttcttgaatggaaatttttaaaacctccttggttaatttctttaagctgggtgttttacccttagcatacaacttcctgaatgggaggtgtcttgaagtgtccctgagtagtgactttgggtgggataacatcaatgcttcgagatcatgcttt

SEQ ID NO: 41 - protein, 5 aa, synthetic construct
  REGION 1..5: note = G4S motif
GGGGS

SEQ ID NO: 42 - protein, 457 aa, Penicillium funiculosum
MLRYLSIVAATAILTGVEAQQSVWGQCGGQGWSGATSCAAGSTCSTLNPYYAQCIPGTATSTTLVKTTSSTSVGTTSPPTTTTTKASTTATTTAAASGNPFSGYQLYANPYYSSEVHTLAIPSLTGSLAAAATKAAEIPSFVWLDTAAKVPTMGTYLANIEAANKAGASPPIAGIFVVYDLPDRDCAAAASNGEYTVANNGVANYKAYIDSIVAQLKAYPDVHTILIIEPDSLANMVTNLSTAKCAEAQSAYYECVNYALIKPHLAHVAMYIDAGHAGWLGWSANLSPAAQLFATVYKNASAPASLRGLATNVANYNAWSISSPPSYTSGDSNYDEKLYINALSPLLTSNGWPDAHFIMDTSRNGVQPTKQQAWGDWCNVIGTGFGVQPTTNTGDPLEDAFVWVKPGGESDGTSNSSATRYDFHCGYSGALQPAPEAGTWFQAYFVQLLTNANPALV

SEQ ID NO: 43 - protein, 408 aa, Rasamsonia emersonii
MVRLSPVLLASIAGSGLPLAQAAGLNTAAKAIGLKYFGTATDNPELSDTAYETQLNNTQDFGQLTPANSMKWDATEPEQNVFTFSAGDQIANLAKANGQMLRCHNLVWYNQLPSWVTSGSWTNETLLAAMKNHITNVVTHYKGQCYAWDVVNEALNDDGTYRSNVFYQYIGEAYIPIAFATAAAADPNAKLYYNDYNIEYPGAKATAAQNLVKLVQSYGARIDGVGLQSHFIVGETPSTSSQQQNMAAFTALGVEVAITELDIRMQLPETEALLTQQATDYQSTVQACANTKGCVGITVWDWTDKYSWVPSTFSGYGDACPWDANYQKKPAYEGILTGLGQTVTSTTYIISPTTSVGTGTTTSSGGSGGTTGVAQHWEQCGGLGWTGPTVCASGYTCTVINEYYSQCL

SEQ ID NO: 44 - protein, 605 aa, Aspergillus niger
MQTLLVSSLVVSLAAALPHYIRSNGIEASLLTDPKDVSGRTVDYIIAGGGLTGLTTAARLTENPNISVLVIESGSYESDRGPIIEDLNAYGDIFGSSVDHAYETVELATNNQTALIRSGNGLGGSTLVNGGTWTRPHKAQVDSWETVFGNEGWNWDNVAAYSLQAERARAPNAKQIAAGHYFNASCHGVNGTVHAGPRDTGDDYSPIVKALMSAVEDRGVPTKKDFGCGDPHGVSMFPNTLHEDQVRSDAAREWLLPNYQRPNLQVLTGQYVGKVLLSQNGTTPRAVGVEFGTHKGNTHNVYAKHEVLLAAGSAVSPTILEYSGIGMKSILEPLGIDTVVDLPVGLNLQDQTTATVRSRITSAGAGQGQAAWFATFNETFGDYSEKAHELLNTKLEQWAEEAVARGGFHNTTALLIQYENYRDWIVNHNVAYSELFLDTAGVASFDVWDLLPFTRGYVHILDKDPYLHHFAYDPQYFLNELDLLGQAAATQLARNISNSGAMQTYFAGETIPGDNLAYDADLSAWTEYIPYHFRPNYHGVGTCSMMPKEMGGVVDNAARVYGVQGLRVIDGSIPPTQMSSHVMTVFYAMALKISDAILEDYASMQ

SEQ ID NO: 45 - protein, 291 aa, Thermomyces lanuginosus
MRSSLVLFFLSAWTALARPVRRAVPQDLLDQFELFSQYSAAAYCAANNHAPVGSDVTCSENVCPEVDAADATFLYSFEDSGLGDVTGLLALDNTNKLIVLSFRGSRSVENWIANLAADLTEISDICSGCEGHVGFVTSWRSVADTIREQVQNAVNEHPDYRVVFTGHSLGGALATIAAAALRGNGYNIDVFSYGAPRVGNRAFAEFLTAQTGGTLYRITHTNDIVPRLPPRDWGYSHSSPEYWVTSGNDVPVTANDITVVEGIDSTDGNNQGNIPDIPSHLWYFGPISECD

SEQ ID NO: 46 - protein, 146 aa, Sus scrofa
MKFLVLAVLLTVGAAQEGISSRALWQFRSMIKCAIPGSHPLMDFNNYGCYCGLGGSGTPVDELDRCCETHDNCYRDAKNLDSCKFLVDNPYTESYSYSCSNTEITCNSKNNACEAFICNCDRNAAICFSKAPYNKEHKNLDTKKYC

SEQ ID NO: 47 - protein, 150 aa, Streptomyces vialaceoruber
MRTTTRTRTTLAAVGAALALGVAAAPPQAAPADKPQVLASFTQTSASSQNAWLAANRNQSAWAAYEFDWSTDLCSQAPDNPFGFPFNTACARHDFGYRNYKAAGSFDANKSRIDSAFYEDMKRVCTGYTGEKNTACNSTAWTYYQAVKIL

SEQ ID NO: 48 - protein, 295 aa, Aspergillus niger
MFSLARLGTVAGLFLLAQAAPASLRRDVSSSLLNNLDLFAQYSAAAYCDENLNSTGTKLTCSVGNCPLVEAASTQSLDEFNESSSYGNPAGYLAADETNKLLVLSFRGSADLANWVANLNFGLEDASDLCSGCEVHSGFWKAWSEIADTITSKVESALSDHSDYSLVLTGHSYGAALAALAATALRNSGHSVELYNYGQPRLGNEALATYITDQNKGGNYRVTHTNDIVPKLPPTLLGYHHFSPEYYISSADEATVTTTDVTEVTGIDATGGNDGTDGTSIDAHRWYFIYISECS

SEQ ID NO: 49 - protein, 515 aa, synthetic construct
  REGION 1..515: note = Mutated glucoamylase
MIRLTVFLTAVFAAVASCVPVELDKRNTGHFQAYSGYTVNRSNFTQWIHEQPAVSWYYLLQNIDYPEGQFKSAKPGVVVASPSTSEPDYFYQWTRDTAITFLSLIAEVEDHSFSNTTLAKVVEYYISNTYTLQRVSNPSGNFDSPNHDGLGEPKFNVDDTAYTASWGRPQNDGPALRAYAISRYLNAVAKHNNGKLLLAGQNGIPYSSASDIYWKIIKPDLQHVSTHWSTSGFDLWEENQGTHFFTALVQLKALSYGIPLSKTYNDPGFTSWLEKQKDALNSYINSSGFVNSGKKHIVESPQLSSRGGLDSATYIAALITHDIGDDDTYTPFNVDNSYVLNSLYYLLVDNKNRYKINGNYKAGAAVGRYPEDVYNGVGTSEGNPWQLATAYAGQTFYTLAYNSLKNKKNLVIEKLNYDLYNSFIADLSKIDSSYASKDSLTLTYGSDNYKNVIKSLLQFGDSFLKVLLDHIDDNGQLTEEINRYTGFQAGAVSLTWSSGSLLSANRARNKLIELL

SEQ ID NO: 50 - protein, 652 aa, synthetic construct
  REGION 1..652: note = Mutated alpha-amylase
MLLQAFLFLLAGFAAKISAGPAAANAETANKSNNVTASSVKNGTILHAWNWSFNTLTQNMKDIRDAGYAAIQTSPINQVKEGNQGDKSMRNWYWLYQPTSYQIGNRYLGTEQEFKDMCAAAEKYGVKVIVDAVINHTTSDYGAISDEIKRIPNWTHGNTQIKNWSDRWDVTQNSLLGLYDWNTQNTEVQVYLKRFLERALNDGADGFRYDAAKHIELPDDGNYGSQFWPNITNTSAEFQYGEILQDSASRDTAYANYMNVTASNYGHSIRSALKNRNLSVSNISHYASDVSADKLVTWVESHDTYANDDEESTWMSDDDIRLGWAVIGSRSGSTPLFFSRPEGGGNGVRFPGKSQIGDRGSALFKDQAITAVNTFHNVMAGQPEELSNPNGNNQVFMNQRGSKGVVLANAGSSSVTINTSAKLPDGRYDNRAGAGSFQVANGKLTGTINARSAAVLYPDDIGNAPHVFLENYQTGAVHSFNDQLTVTLRANAKTTKAVYQINNGQQTAFKDGDRLTIGKGDPIGTTYNIKLTGTNGEGAARTQEYTFVKKDPSQTNIIGYQNPDHWGQVNAYIYKHDGGRAIELTGSWPGKAMTKNANGMYTLTLPENTDTANAKVIFNNGSAQVPGQNQPGFDYVQNGLYNNSGLNGYLPH

SEQ ID NO: 51 - protein, 713 aa, synthetic construct
  REGION 1..713: note = Mutated maltogenic alpha-amylase
MLLQAFLFLLAGFAAKISAYNPNAAEASSSASVKGDVIYQIIIDRFYDGDTTNNNPAKSYGLYDPTKSKWKMYWGGDLEGVRQKLPYLKQLGVTTIWLSPVLDNLDTLAGTDNTGYHGYWTRDFKQIEEHFGNWTTFDTLVNDAHQNGIKVIVDFVPNHSTPFKANDSTFAEGGALYNNGTYMGNYFDDATKGYFHHNGDISNWDDRYEAQWKNFTDPAGFSLADLSQENGTIAQYLTDAAVQLVAHGADGLRIDAVKHFNSGFSKSLADKLYQKKDIFLVGEWYGDDPGTANHLEKVRYANNSGVNVLDFDLNTVIRNVFGTFTQTMYDLNNMVNQTGNEYKYKENLITFIDNHDMSRFLSVNSNKANLHQALAFILTSRGTPSIYYGTEQYMAGGNDPYNRGMMPAFDTTTTAFKEVSTLAGLRRNNAAIQYGTTTQRWINNDVYIYERKFFNDVVLVAINRNTQSSYSISGLQTALPNGSYADYLSGLLGGNGISVSNGSVASFTLAPGAVSVWQYSTSASAPQIGSVAPNMGIPGNVVTIDGKGFGTTQGTVTFGGVTATVKSWTSNRIEVYVPNMAAGLTDVKVTAGGVSSNLYSYNILSGTQTSVVFTVKSAPPTNLGDKIYLTGNIPELGNWSTDTSGAVNNAQGPLLAPNYPDWFYVFSVPAGKTIQFKFFIKRADGTIQWENGSNHVATTPTGATGNITVTWQN

SEQ ID NO: 52 - protein, 19 aa, Saccharomyces cerevisiae
MLLQAFLFLLAGFAAKISA

SEQ ID NO: 53 - protein, 22 aa, synthetic construct
  REGION 1..22: note = HA tag
KDNSSTIEGRYPYDVPDYALQA

SEQ ID NO: 54 - protein, 18 aa, synthetic construct
  REGION 1..18: note = Modified G4S linker
SGGGGSGGGGSGGGGSAS

SEQ ID NO: 55 - DNA, 750 bp, synthetic construct
  misc_feature 1..750: note = Promoter of trx2 gene
  source 1..750: mol_type = other DNA
ataaccacaatgatcgcagaccgtcgacatgataatgacttctttaaagtgtgggatatttactggcttcatatgagtttcacactcttgggtacacgatggacaagaagctctgaatgtttgcacctcgttgttaaagttttcgatgtcggtggcgtctgacaaaaactgtgggtttgctgagccaactttgacagattcagaaggatttctttcacggttggccaattgttttaattgttcttggcgacgttgctccaactggtctctagtaataatgccaacttgaacgttttgttcgtcggttctcacgtactgggtatgagaccatttgtgttgaggttcaccgggtttgtattcgatccaggaatttcccgcaggatcatccaaaataaatgtaatcggaatagtgttgggttcacaattgatgtaggatttaactttctgtacgaagtcatcgatcttcttgtaaagagcttcgtctatagattttctcatttcctggtcttgcgacagatcgtcgatcatctcggataacaaaccttcaactgtcgtcaattgacctctcttagcaggaatctcaatgtctagctcgacaaacttacaagtggcagtttctgacttaataacttgcctgttaaaatcttcacggcactccactttcaaaacgtaacgagagcccttctcttgaatttgagaagcgggttggatctcacagttcttaaacccacagtgaggacagtcgaatga

SEQ ID NO: 56 - DNA, 750 bp, synthetic construct
  misc_feature 1..750: note = Promoter of sti1 gene
  source 1..750: mol_type = other DNA
taccacaaagggtaaaacgtcaataaaagcaagcaatgttattcgtgccagagaactatatctggcgtacgtcttatatataacacaagcaagggcaaatacgtggttagtggtgtaaaaactgaagggattaatttacatacaactagatccatctttctcaaaaatgacttcagtatcgccctcgccacctgccagtcgatcgggctcaatgtgctccgacttaccgtcctctttgcagactgagaaactggcacatattataggtcttgatgccgacgatgaagttctccggcgcgtaaccaagcagttgagcagatctaggagaattgcttgtctgactggggcaggcatttcgtgcaacgcgggcattcctgactttcgctcttctgatgggctctacgacctagtgaaaaaggattgttcacagtattggtctatcaagtccggcagggaaatgtttgatatttcgctatttagagatgacttcaaaatatccatttttgctaaatttatggagaggctctattcaaatgttcaattggcaaagccgactaagacgcacaagttcattgcgcatctaaaagataggaacaaactgctgcgctgttacacgcaaaacatcgatgggctcgaagaaagcataggacttactttatcaaataggaaattaccgcttacctcatttagttcacattggaaaaatctggatgtcgttcagttgcacggcgacctgaaaactctttcgtg

SEQ ID NO: 57 - DNA, 750 bp, synthetic construct
  misc_feature 1..750: note = Promoter of gdp1 gene
  source 1..750: mol_type = other DNA
aaggaaaatatatactctttcccaggcaaggtgacagcggtccccgtctcctccacaaaggcctctcctggggtttgagcaagtctaagtttacgtagcataaaaattctcggattgcgtcaaataataaaaaaagtaactccacttctacttctacatcggaaaaacattccattcacatatcgtctttggcctatcttgttttgtccttggtagatcaggtcagtacaaacgcaacacgaaagaacaaaaaaagaagaaaaacagaaggccaagacagggtcaatgagactgttgtcctcctactgtccctatgtctctggccgatcacgcgccattgtccctcagaaacaaatcaaacacccacaccccgggcacccaaagtccccacccacaccaccaatacgtaaacggggcgccccctgcaggccctcctgcgcgcggcctcccgccttgcttctctcccctcccttttctttttccagttttccctattttgtccctttttccgcacaacaagtatcagaatgggttcatcaaatctatccaacctaattcgcacgtagactggcttggtattggcagtttcgcagttatatatatactaccatgagtgaaactgttacgttaccttaaattctttctccctttaattttcttttatcttactctcctacataagacatcaagaaacaattgtatattgtacacccccccccctccacaaacacaaatattgataatataaag

SEQ ID NO: 58 - DNA, 750 bp, synthetic construct
  misc_feature 1..750: note = Promoter of cup1 gene
  source 1..750: mol_type = other DNA
taaatatatgctgagatttagcaagaaaaaacaaaattttgcgagaaactctgataacaataatgttacagattatagtcagtcggcgaagaacaaaaatgttctcttgaaattccccgttagtgaactgaacagaatctatttaaaatttaaggagatttcagattttttaatggaaagagaagttgtccaaaggagtataattattgacaaggatttggaatctgataatctgggtattactacggcaaacttcaacgatttctatgatgcattttataattagtaagccgatcccattaccgacatttgggcgctatacgtgcatatgttcatgtatgtatctgtatttaaaacacttttgtattatttttcctcatatatgtgtataggtttatacggatgatttaattattacttcaccaccctttatttcaggctgatatcttagccttgttactagttagaaaaagacatttttgctgtcagtcactgtcaagagattcttttgctggcatttcttctagaagcaaaaagagcgatgcgtcttttccgctgaaccgttccagcaaaaaagactaccaacgcaatatggattgtcagaatcatataaaagagaagcaaataactccttgtcttgtatcaattgcattataatatcttcttgttagtgcaatatcatatagaagtcatcgaaatagatattaagaaaaacaaactgtacaatcaatcaatcaatcatcacataaa

SEQ ID NO: 59 - DNA, 750 bp, synthetic construct
  misc_feature 1..750: note = Promoter of glo1 gene
  source 1..750: mol_type = other DNA
tattaatccaaaaagtgaatctttgacacccctttctcctatcttgcttagtaccgagtgatcttttgcataatcaaaacaagtgaagaaggtcgagttttgaaccttctctaatataagtcgacggtctttcgtgatggcgtcaatattacttagtcttttgtacttcacatataccattaatggcgtcaatcccttataattttcctcattaatatctagcttagtcagttgtaaaaggattggaatgtttgttttcaaaacatgcaacaagctattgcccttattatcggtgtggtctagatagtcaaacaaactgttgtgctttctataccaagtatttgcgatatcaaatgcggtcttcaccatttcttcataatttggttgatcataacttctaaagatggaaaataaaggcgtttgtccactggagttttttcgtttccaatcaatataatttccgatgcttttaagtatatccatttcatgggttagataatgagccacggtacgtgcatatttatctgttttattgatataagaaaccagctcctcttcagtacaattgaacagcatgatctttatgagaactttcgcggcttctaaatttcctgcttttatcgattctataagcagcgtagaaccatcaatcgtttcgtcctctaaaaggtcttctactggaaagtcgttttcatattcagaaagaatatctaataagatgtagtttttatgatttgttatacatatgga

SEQ ID NO: 60 - DNA, 750 bp, synthetic construct
  misc_feature 1..750: note = Promoter of ctt1 gene
  source 1..750: mol_type = other DNA
ttaactgcaaagacccgtcacctatgaataagatgactctcttgttggggtcaatctcctcagcggcaaaggcagcacctaaagttgctcctgttgtaaaaccgatagacccccacaacacttgcgagataccgtaggcgtccttaggaaagatagtttgattgataccgaaggcagacgtgccggtctcggaaatgataacatcaccttcttgcaagaacttggacaattcgttccacaaccactcttgtttcaagggcgtgctagcagatacacctttgtttgcgggagttttggttggtacgggaacgctcttgtagcccttaataacatcgggaataaccttcagtaagttttgtagtgcaaatttcatttgtacgccggggaacgtagcgttcttcacctttacgtaatcggaatgaaactccactacatttttagtcttgtaggagtaggaaaacgaacctgtgttaaaatcagagagcaaagcaccgaccgaaaggatcaaatcagccgactcaacggcctgtttcacgtctggtttggacagcgttcccacataaacaccgccatatctgggatgctgttcatctattgaccctttacctaaaggtgtcacaaaagctgggaattgcgtcaaatcaattaacttctgggtttcctttttaacgttgtgcctagaagcacaggcatccgatagtatgacagggtttttcgaattctggatcaattctagtacggtatcaataa

SEQ ID NO: 61 - DNA, 750 bp, synthetic construct
  misc_feature 1..750: note = Promoter of ygp1 gene
  source 1..750: mol_type = other DNA
tctcataattggtcagaagaaaggaaatctaggcaattgagttctttgggtaaaaaagagtcacaatttttaaggctgcgtagaacgagattatcgttagaagatttccacactgtgaaagtcattggaaaaggggcatttggtgaagtcagactggttcagaagaaagacaccggaaaaatatatgcaatgaaaactttattaaaatccgaaatgtacaaaaaggaccaattagcacacgtcaaggctgaaagggatgttctggctggaagtgattctccatgggtggtttcgctatattactcattccaagatgctcaatacttatatttaatcatggaatttttgcccggtggtgatttgatgaccatgctaatcaggtggcaactatttacagaggatgttactagattttacatggctgagtgtattttggccatcgaaaccattcataaattaggattcattcacagagatattaaaccagataatattttgatcgatattagaggtcatataaaattatctgatttcgggttgtctacggggttccataaaactcacgactcaaactactataaaaagcttttgcaacaagatgaggcaactaatggtatttccaagccaggtacttacaatgcaaatacaaccgatactgcaaataaaaggcaaacaatggttgtggattctattagtctaacaatgtcaaacaggcaacaaattcagacatggagaaaatcacgtcgttta

SEQ ID NO: 62 - DNA, 750 bp, synthetic construct
  misc_feature 1..750: note = Promoter of gsy2 gene
  source 1..750: mol_type = other DNA
tattatagctcttgataacaatgaaatttcaacaattattcactcaaccctcaagtgtatatcgccaagatcctaatcacccctctctggtggccttccctcattgtttttacacagaacaagaatccataaaatcaagatattgggaacaattcattgtcttaggaacaagtttttataatttagtttcattagcctattgtaacttcttgtttttttttttattttggctggcaaaacaagaagtataaagaagttaccactgctataacgtatatcttaaatcaagtgggcaattcttcgaataaacttagaggcgctgaagaaagaaccgctcaattagttcgatcatacaaaatacagatattgcgctgtgtattatcattacagaaagtgtgatataaacaatgctgtgttgtattcggtcttttttttccgcctgcagattgtcgtttttgtttttttttctcgtgtagctgcagttatcatcgttttgcatgtctgttctgtcggtgaagccgatctcatggcacttcgctttgataccgtaaagaatcttcttcattaatacggcactgcaaggcgatatctatctctggggttaggactgataaataggtacttatcagttatcactagagacgaactgtttacgttttgaagctcgacagcaggggttcttaacgggcgtcggcctagacctcaccttgcgagaaatttttagttcatatccaggggatggtgaatggt

SEQ ID NO: 63 - DNA, 750 bp, synthetic construct
  misc_feature 1..750: note = Promoter of hsp12 gene
  source 1..750: mol_type = other DNA
gcttgtccacaatcaccatggggttatattgcattatttttttatcttcgttatcattccatactgtggcttcattccagtattttatgagtttgctgaaggattcgggggtaatagtgcccacggtggtcaaaacctttagcgtctcagtgacctgttccaaatccccctcttccattcgccttatataaaatccatcgggtaagctcattattttatgttgatatccagcttccgttcgtcaactattctctcgagctcagttttgggttttggcatgtaaacaatgccttcgcttgtattacgcaaaaaaaaaaaaaataaataaaaaaaaaaaaaaaaaaataaggtataaatcgttggttcttttatgcacaattatttaactatagttatctatttacgtaaaggcttctatttttccttatctacaagaaattgcatgaagtttaattttttttgtcacctttgatcttcctgaatgtgttggtaatgaaattttctagtctcttcaaagtgttgtcgtcatccttttttgcgtgtttttcctcttcttgtttttgtttcttcagtatctcttcattaatggctgtacccgcggctgtgcccggttgcatggttttcttggccatgtcatcgttggtgacatctgccagtgcctcccacaagcatttttctgccagcgattgcggtttcttaacaacgatcttgtactggactttcatatcaccgcgaatggttgatgtttta

SEQ ID NO: 64 - DNA, 750 bp, synthetic construct
  misc_feature 1..750: note = Promoter of mol1/thi4 genes
  source 1..750: mol_type = other DNA
tcgttgaaagttctagatttgggtacggaagcagccatgtaaatggtcttcctttgtaataatatcgtcactggagtttttaaattagagtacggattcaagttaacgaaaaatttctgttggtatctgatagcaatttgtcgacaaggtggagagtttttgaagtttttttttgtaacagttatgttacactatttaccagagaaacaccaagacaggagccctcagaagctttcgtgttgtcagaacataaatatcttctatatgttttattcttttatattaatcaatattttatgttaaatcatattattattcgttaatgcttaacttgccctatttcaaaatcggaagggtagtatggtgacaagcggtgtttttggtgtatgtttactgctaagagtataccgtcctgtttacttttttaccttttgttccgttattgatttttcgcagcaaggttgaagcttccatatttgaaaatgaaattaagaagtagagatgaaaaacagcgacgaaattactttttatagcttctttcccttctgactccgttttataaacaggggatctttaagggcttacaaaataaatataaacactaacacatatatattattcgacctacagtttttgcgaccaatgaagtttacctattttgagatggtgcttacgtagtttgcttaaggtcaaggcgggattaagcttgcgctttctctaaataatatcatatgttacagacagggataa

SEQ ID NO: 65 - protein, 695 aa, Geobacillus stearothermophilus
MYNPNAAEASSSASVKGDVIYQIIIDRFYDGDTTNNNPAKSYGLYDPTKSKWKMYWGGDLEGVRQKLPYLKQLGVTTIWLSPVLDNLDTLAGTDNTGYHGYWTRDFKQIEEHFGNWTTFDTLVNDAHQNGIKVIVDFVPNHSTPFKANDSTFAEGGALYNNGTYMGNYFDDATKGYFHHNGDISNWDDRYEAQWKNFTDPAGFSLADLSQENGTIAQYLTDAAVQLVAHGADGLRIDAVKHFNSGFSKSLADKLYQKKDIFLVGEWYGDDPGTANHLEKVRYANNSGVNVLDFDLNTVIRNVFGTFTQTMYDLNNMVNQTGNEYKYKENLITFIDNHDMSRFLSVNSNKANLHQALAFILTSRGTPSIYYGTEQYMAGGNDPYNRGMMPAFDTTTTAFKEVSTLAGLRRNNAAIQYGTTTQRWINNDVYIYERKFFNDVVLVAINRNTQSSYSISGLQTALPNGSYADYLSGLLGGNGISVSNGSVASFTLAPGAVSVWQYSTSASAPQIGSVAPNMGIPGNVVTIDGKGFGTTQGTVTFGGVTATVKSWTSNRIEVYVPNMAAGLTDVKVTAGGVSSNLYSYNILSGTQTSVVFTVKSAPPTNLGDKIYLTGNIPELGNWSTDTSGAVNNAQGPLLAPNYPDWFYVFSVPAGKTIQFKFFIKRADGTIQWENGSNHVATTPTGATGNITVTWQN

SEQ ID NO: 66 - protein, 411 aa, Citrobacter braakii
EEQNGMKLERVVIVSRHGVRAPTKFTPIMKDVTPDQWPQWDVPLGWLTPRGGELVSELGQYQRLWFTSKGLLNNQTCPSPGQVAVIADTDQRTRKTGEAFLAGLAPKCQIQVHYQKDEEKNDPLFNPVKMGKCSFNTLKVKNAILERAGGNIELYTQRYQSSFRTLENVLNFSQSETCKTTEKSTKCTLPEALPSEFKVTPDNVSLPGAWSLSSTLTEIFLLQEAQGMPQVAWGRITGEKEWRDLLSLHNAQFDLLQRTPEVARSRATPLLDMIDTALLTNGTTENRYGIKLPVSLLFIAGHDTNLANLSGALDLKWSLPGQPDNTPPGGELVFEKWKRTSDNTDWVQVSFVYQTLRDMRDIQPLSLEKPAGKVDLKLIACEEKNSQGMCSLKSFSRLIKEIRVPECAVTE

SEQ ID NO: 67 - protein, 410 aa, Escherichia coli
QSEPELKLESVVIVSRHGVRAPTKATQLMQDVTPDAWPTWPVKLGWLTPRGGELIAYLGHYQRQRLVADGLLAKKGCPQSGQVAIIADVDERTRKTGEAFAAGLAPDCAITVHTQADTSSPDPLFNPLKTGVCQLDNANVTDAILSRAGGSIADFTGHRQTAFRELERVLNFPQSNLCLKREKQDESCSLTQALPSELKVSADNVSLTGAVSLASMLTEIFLLQQAQGMPEPGWGRITDSHQWNTLLSLHNAQFYLLQRTPEVARSRATPLLDLIKTALTPHPPQKQAYGVTLPTSVLFIAGHDTNLANLGGALELNWTLPGQPDNTPPGGELVFERWRRLSDNSQWIQVSLVFQTLQQMRDKTPLSLNTPPGEVKLTLAGCEERNAQGMCSLAGFTQIVNEARIPACSL

SEQ ID NO: 68 - protein, 19 aa, Saccharomyces cerevisiae
MLLQAFLFLLAGFAAKISA

SEQ ID NO: 69 - protein, 18 aa, Saccharomyces cerevisiae
MQLLRCFSIFSVIASVLA

SEQ ID NO: 70 - DNA, 500 bp, Saccharomyces cerevisiae
  source 1..500: mol_type = genomic DNA
tagcgtgttacgcacccaaactttttatgaaagtctttgtttataatgatgaggtttataaatatatagtggagcaaagattaatcactaaatcaagaagcagtaccagtattttttttatatcaagtagtgataatggaaatagcccaaatttggcttccgtcggcacatagcacgtttgagagacattatcaccatcaagcatcgagccgcccaaacctaactgtataagttttttcacgtttttgatttttccttgcacacttcgatattactctcacgataaaagggccgaagagaatatttttcttgaacatccagaattttaattcggagaaatttcacaagccgccgatttaagggtcctgtgttcttaataatcagcctctctcaaagcaggtaagaggcagtctttcttttaacaataggagacattcgaactaaaacatcagccccaaaaatgcgcttgaaggtcattaggatttggatttcttcctcat

SEQ ID NO: 71 - protein, 460 aa, Pyrococcus furiosus
MNIKKLTPLLTLLLFFIVLASPVSAAKYLELEEGGVIMQAFYWDVPGGGIWWDHIRSKIPEWYEAGISAIWLPPPSKGMSGGYSMGYDPYDYFDLGEYYQKGTVETRFGSKEELVRLIQTAHAYGIKVIADVVINHRAGGDLEWNPFVGDYTWTDFSKVASGKYTANYLDFHPNELHCCDEGTFGGFPDICHHKEWDQYWLWKSNESYAAYLRSIGFDGWRFDYVKGYGAWVVRDWLNWWGGWAVGEYWDTNVDALLSWAYESGAKVFDFPLYYKMDEAFDNNNIPALVYALQNGQTVVSRDPFKAVTFVANHDTDIIWNKYPAYAFILTYEGQPVIFYRDFEEWLNKDKLINLIWIHDHLAGGSTTIVYYDNDELIFVRNGDSRRPGLITYINLSPNWVGRWVYVPKFAGACIHEYTGNLGGWVDKRVDSSGWVYLEAPPHDPANGYYGYSVWSYCGVG

SEQ ID NO: 72 - protein, 457 aa, Thermococcus hydrothermalis
MARKVLVALLVFLVVLSVSAVPAKAETLENGGVIMQAFYWDVPGGGIWWDTIAQKIPDWASAGISAIWIPPASKGMSGGYSMGYDPYDFFDLGEYYQKGSVETRFGSKEELVNMINTAHAHNMKVIADIVINHRAGGDLEWNPFTNSYTWTDFSKVASGKYTANYLDFHPNELHAGDSGTFGGYPDICHDKSWDQHWLWASNESYAAYLRSIGIDAWRFDYVKGYAPWVVKNWLNRWGGWAVGEYWDTNVDALLSWAYDSGAKVFDFPLYYKMDEAFDNNNIPALVDALKNGGTVVSRDPFKAVTFVANHDTNIIWNKYPAYAFILTYEGQPAIFYRDYEEWLNKDRLRNLIWIHDHLAGGSTDIIYYDSDELIFVRNGYGDKPGLITYINLGSSKAGRWVYVPKFAGSCIHEYTGNLGGWIDKWVDSSGRVYLEAPAHDPANGQYGYSVWSYCGVG

SEQ ID NO: 73 - DNA, 390 bp, synthetic construct
  misc_feature 1..390: note = SPI1 tethering moiety
  source 1..390: mol_type = other DNA
  CDS 1..390
ttggtatctaattctagttcctctgtaatcgtggtaccatcaagcgatgctactattgccggtaacgatacagccacgccagcaccagagccatcatccgccgctccaatattctacaactcgactgctactgcaacacagtacgaagttgtcagtgaattcactacttactgcccagaaccaacgactttcgtaacgaatggcgctacattcactgttactgccccaactacgttaacaattaccaactgtccttgcactatcgagaagcctacttcagaaacatcggtttcttctacacatgatgtggagacaaattctaatgctgctaacgcaagagcaatcccaggagccctaggtttggctggtgcagttatgatgcttttatga

SEQ ID NO: 74 - protein, 129 aa, synthetic construct
  REGION 1..129: note = Synthetic Construct
LVSNSSSSVIVVPSSDATIAGNDTATPAPEPSSAAPIFYNSTATATQYEVVSEFTTYCPEPTTFVTNGATFTVTAPTTLTITNCPCTIEKPTSETSVSSTHDVETNSNAANARAIPGALGLAGAVMMLL

SEQ ID NO: 75 - DNA, 66 bp, synthetic construct
  misc_feature 1..66: note = 21aa-truncation of the SPI1 tethering moiety
  source 1..66: mol_type = other DNA
  CDS 1..66
gctgctaacgcaagagcaatcccaggagccctaggtttggctggtgcagttatgatgcttttatga

SEQ ID NO: 76 - protein, 21 aa, synthetic construct
  REGION 1..21: note = Synthetic Construct
AANARAIPGALGLAGAVMMLL

SEQ ID NO: 77 - DNA, 156 bp, synthetic construct
  misc_feature 1..156: note = 51aa-truncation of the SPI1 tethering moiety
  source 1..156: mol_type = other DNA
  CDS 1..156
ttaacaattaccaactgtccttgcactatcgagaagcctacttcagaaacatcggtttcttctacacatgatgtggagacaaattctaatgctgctaacgcaagagcaatcccaggagccctaggtttggctggtgcagttatgatgcttttatga

SEQ ID NO: 78 - protein, 51 aa, synthetic construct
  REGION 1..51: note = Synthetic Construct
LTITNCPCTIEKPTSETSVSSTHDVETNSNAANARAIPGALGLAGAVMMLL

SEQ ID NO: 79 - DNA, 246 bp, synthetic construct
  misc_feature 1..246: note = 81aa-truncation of the SPI1 tethering moiety
  source 1..246: mol_type = other DNA
  CDS 1..246
gaagttgtcagtgaattcactacttactgcccagaaccaacgactttcgtaacgaatggcgctacattcactgttactgccccaactacgttaacaattaccaactgtccttgcactatcgagaagcctacttcagaaacatcggtttcttctacacatgatgtggagacaaattctaatgctgctaacgcaagagcaatcccaggagccctaggtttggctggtgcagttatgatgcttttatga

SEQ ID NO: 80 - protein, 81 aa, synthetic construct
  REGION 1..81: note = Synthetic Construct
EVVSEFTTYCPEPTTFVTNGATFTVTAPTTLTITNCPCTIEKPTSETSVSSTHDVETNSNAANARAIPGALGLAGAVMMLL

SEQ ID NO: 81 - DNA, 336 bp, synthetic construct
  misc_feature 1..336: note = 111aa-truncation of the SPI1 tethering moiety
  source 1..336: mol_type = other DNA
  CDS 1..336
attgccggtaacgatacagccacgccagcaccagagccatcatccgccgctccaatattctacaactcgactgctactgcaacacagtacgaagttgtcagtgaattcactacttactgcccagaaccaacgactttcgtaacgaatggcgctacattcactgttactgccccaactacgttaacaattaccaactgtccttgcactatcgagaagcctacttcagaaacatcggtttcttctacacatgatgtggagacaaattctaatgctgctaacgcaagagcaatcccaggagccctaggtttggctggtgcagttatgatgcttttatga

SEQ ID NO: 82 - protein, 111 aa, synthetic construct
  REGION 1..111: note = Synthetic Construct
IAGNDTATPAPEPSSAAPIFYNSTATATQYEVVSEFTTYCPEPTTFVTNGATFTVTAPTTLTITNCPCTIEKPTSETSVSSTHDVETNSNAANARAIPGALGLAGAVMMLL

SEQ ID NO: 83 - DNA, 339 bp, synthetic construct
  misc_feature 1..339: note = CCW12 tethering moiety
  source 1..339: mol_type = other DNA
  CDS 1..339
gttaccactgctactgtcagccaagaatctaccactttggtcaccatcacttcttgtgaagaccacgtctgttctgaaactgtctccccagctttggtttccaccgctaccgtcaccgtcgatgacgttatcactcaatacaccacctggtgcccattgaccactgaagccccaaagaacggtacttctactgctgctccagttacctctactgaagctccaaagaacaccacctctgctgctccaactcactctgtcacctcttacactggtgctgctgctaaggctttgccagctgctggtgctttgttggctggtgccgctgctttgttgttgtaa

SEQ ID NO: 84 - protein, 112 aa, synthetic construct
  REGION 1..112: note = Synthetic Construct
VTTATVSQESTTLVTITSCEDHVCSETVSPALVSTATVTVDDVITQYTTWCPLTTEAPKNGTSTAAPVTSTEAPKNTTSAAPTHSVTSYTGAAAKALPAAGALLAGAAALLL

SEQ ID NO: 85 - DNA, 75 bp, synthetic construct
  misc_feature 1..75: note = 24aa-truncation of the CCW12 tethering moiety
  source 1..75: mol_type = other DNA
  CDS 1..75
tacactggtgctgctgctaaggctttgccagctgctggtgctttgttggctggtgccgctgctttgttgttgtaa

SEQ ID NO: 86 - protein, 24 aa, synthetic construct
  REGION 1..24: note = Synthetic Construct
YTGAAAKALPAAGALLAGAAALLL

SEQ ID NO: 87 - DNA, 150 bp, synthetic construct
  misc_feature 1..150: note = 49aa-truncation of the CCW12 tethering moiety
  source 1..150: mol_type = other DNA
  CDS 1..150
actgctgctccagttacctctactgaagctccaaagaacaccacctctgctgctccaactcactctgtcacctcttacactggtgctgctgctaaggctttgccagctgctggtgctttgttggctggtgccgctgctttgttgttgtaa

SEQ ID NO: 88 - protein, 49 aa, synthetic construct
  REGION 1..49: note = Synthetic Construct
TAAPVTSTEAPKNTTSAAPTHSVTSYTGAAAKALPAAGALLAGAAALLL

SEQ ID NO: 89 - DNA, 225 bp, synthetic construct
  misc_feature 1..225: note = 74aa-truncation of the CCW12 tethering moiety
  source 1..225: mol_type = other DNA
  CDS 1..225
accgtcgatgacgttatcactcaatacaccacctggtgcccattgaccactgaagccccaaagaacggtacttctactgctgctccagttacctctactgaagctccaaagaacaccacctctgctgctccaactcactctgtcacctcttacactggtgctgctgctaaggctttgccagctgctggtgctttgttggctggtgccgctgctttgttgttgtaa

SEQ ID NO: 90 - protein, 74 aa, synthetic construct
  REGION 1..74: note = Synthetic Construct
TVDDVITQYTTWCPLTTEAPKNGTSTAAPVTSTEAPKNTTSAAPTHSVTSYTGAAAKALPAAGALLAGAAALLL

SEQ ID NO: 91 - DNA, 300 bp, synthetic construct
  misc_feature 1..300: note = 99aa-truncation of the CCW12 tethering moiety
  source 1..300: mol_type = other DNA
  CDS 1..300
gtcaccatcacttcttgtgaagaccacgtctgttctgaaactgtctccccagctttggtttccaccgctaccgtcaccgtcgatgacgttatcactcaatacaccacctggtgcccattgaccactgaagccccaaagaacggtacttctactgctgctccagttacctctactgaagctccaaagaacaccacctctgctgctccaactcactctgtcacctcttacactggtgctgctgctaaggctttgccagctgctggtgctttgttggctggtgccgctgctttgttgttgtaa

SEQ ID NO: 92 - protein, 99 aa, synthetic construct
  REGION 1..99: note = Synthetic Construct
VTITSCEDHVCSETVSPALVSTATVTVDDVITQYTTWCPLTTEAPKNGTSTAAPVTSTEAPKNTTSAAPTHSVTSYTGAAAKALPAAGALLAGAAALLL

SEQ ID NO: 93 - protein, 15 aa, synthetic construct
  REGION 1..15: note = Linker 1
GGGGSGGGGSGGGGS

SEQ ID NO: 94 - protein, 8 aa, synthetic construct
  REGION 1..8: note = Linker 2
GGGGGGGG

SEQ ID NO: 95 - protein, 40 aa, synthetic construct
  REGION 1..40: note = Linker 3
GGGGSGGGGSGGGGSGGGGSGGGGSGGGGSGGGGSGGGGS

SEQ ID NO: 96 - protein, 12 aa, synthetic construct
  REGION 1..12: note = Linker 4
GSAGSAAGSGEF

SEQ ID NO: 97 - protein, 12 aa, synthetic construct
  REGION 1..12: note = Linker 5
EAAKEAAKEAAK

SEQ ID NO: 98 - protein, 20 aa, synthetic construct
  REGION 1..20: note = Linker 6
APAPAPAPAPAPAPAPAPAP

SEQ ID NO: 99 - protein, 46 aa, synthetic construct
  REGION 1..46: note = Linker 7
AEAAAKEAAAKEAAAKEAAAKALEAEAAAKEAAAKEAAAKEAAAKA

SEQ ID NO: 100 - protein, 4 aa, synthetic construct
  REGION 1..4: note = EA2K motif
EAAK

SEQ ID NO: 101 - protein, 5 aa, synthetic construct
  REGION 1..5: note = EA3K motif
EAAAK

SEQ ID NO: 102 - DNA, 1752 bp, Aspergillus niger
  source 1..1752: mol_type = genomic DNA
tccaatggtattgaggcttccttgttgactgatccaaaagatgtttctggtagaaccgtcgattacattattgctggtggtggtttgactggtttaactactgctgctagattgactgaaaacccaaacatctccgttttggttatcgaatctggttcctacgaatctgatagaggtccaattatcgaagatttgaacgcctacggtgatatctttggttcttctgttgatcatgcttacgaaaccgttgaattggctaccaacaatcaaactgccttgattagatctggtaacggtttaggtggttctactttggttaatggtggtacttggactagaccacataaggctcaagttgattcttgggaaactgtttttggtaacgaaggttggaattgggataatgttgctgcttattcattgcaagctgaaagggctagagcaccaaatgctaaacaaattgctgctggtcattacttcaatgcctcttgtcatggtgttaacggtactgttcatgctggtccaagagatactggtgatgattattctccaatcgttaaggctttgatgtccgctgttgaagatagaggtgttccaactaagaaagatttcggttgtggtgatccacatggtgtttctatgtttccaaataccttgcacgaagatcaagttagatctgatgctgcaagagaatggttgttgccaaattatcaaagaccaaacttgcaggtcttgactggtcaatatgttggtaaggttttgttgtcccaaaacggtactactccaagagctgttggtgttgaatttggtactcataagggtaacacccataacgtttacgccaaacatgaagttttgttagctgctggttctgctgtttctccaactattttggaatactccggtatcggtatgaagtccattttggaaccattgggtattgataccgttgttgatttgccagttggtttgaacttacaagatcaaactaccgctaccgtcagatctagaattacttctgctggtgctggtcaaggtcaagctgcttggtttgctacttttaacgaaactttcggtgactactctgaaaaggcccatgaattattgaacaccaaattggaacaatgggctgaagaggctgttgctagaggtggttttcataacactactgccttgttgatccagtacgaaaattacagagattggatcgttaaccacaacgttgcttactctgagttgtttttggatactgctggtgttgcttcttttgatgtatgggatttgttgccattcaccagaggttacgttcacattttggataaggatccatacttgcatcatttcgcttacgacccacaatactttttgaacgaattggacttgttgggtcaagccgctgctactcaattggctagaaacatttctaattccggtgctatgcaaacctatttcgctggtgaaactattccaggtgataacttggcttatgatgctgatttgtctgcttggactgagtacattccataccatttcagaccaaattaccacggtgttggtacttgttctatgatgccaaaagaaatgggtggtgttgttgataatgcagctagagtttacggtgttcaaggtttgagagttatcgatggttctattccaccaactcaaatgtcctctcatgttatgactgttttctacgctatggccttgaagatttccgatgcaattttggaagattacgcctccatgcaataa

SEQ ID NO: 103 - protein, 583 aa, Aspergillus niger
SNGIEASLLTDPKDVSGRTVDYIIAGGGLTGLTTAARLTENPNISVLVIESGSYESDRGPIIEDLNAYGDIFGSSVDHAYETVELATNNQTALIRSGNGLGGSTLVNGGTWTRPHKAQVDSWETVFGNEGWNWDNVAAYSLQAERARAPNAKQIAAGHYFNASCHGVNGTVHAGPRDTGDDYSPIVKALMSAVEDRGVPTKKDFGCGDPHGVSMFPNTLHEDQVRSDAAREWLLPNYQRPNLQVLTGQYVGKVLLSQNGTTPRAVGVEFGTHKGNTHNVYAKHEVLLAAGSAVSPTILEYSGIGMKSILEPLGIDTVVDLPVGLNLQDQTTATVRSRITSAGAGQGQAAWFATFNETFGDYSEKAHELLNTKLEQWAEEAVARGGFHNTTALLIQYENYRDWIVNHNVAYSELFLDTAGVASFDVWDLLPFTRGYVHILDKDPYLHHFAYDPQYFLNELDLLGQAAATQLARNISNSGAMQTYFAGETIPGDNLAYDADLSAWTEYIPYHFRPNYHGVGTCSMMPKEMGGVVDNAARVYGVQGLRVIDGSIPPTQMSSHVMTVFYAMALKISDAILEDYASMQ

SEQ ID NO: 104 - DNA, 1437 bp, Aspergillus oryzae
  source 1..1437: mol_type = genomic DNA
gctactccagctgattggagatcacaatctatctactttttgttgaccgacagattcgctagaactgatggttctactactgctacttgtaataccgctgatagaaagtattgtggtggtacttggcaaggtatcatcgataagttggattacattcaaggtatgggtttcaccgctatttggattactccagttactgctcaattgccacaaactactgcttatggtgatgcttatcatggttattggcaacaggatatctactccttgaacgaaaattacggtactgccgatgatttgaaggctttgtcatctgctttacatgaacgtggtatgtacttgatggttgatgttgttgctaaccacatgggttatgatggtgctggttcttctgttgattactctgtttttaagcccttcagctcccaagattactttcatccattctgcttgatccaaaactacgaagatcaaactcaagtcgaagattgctggttgggtgataatactgtttctttgccagatttggataccaccaaggatgttgttaagaacgaatggtatgattgggtcggttctttggtttccaactactctattgatggtttgagaatcgataccgtcaagcacgttcaaaaagatttttggccaggttacaacaaagctgctggtgtttactgtattggtgaagttttagatggtgatccagcttacacttgtccataccaaaatgttatggatggcgttttgaactacccaatctactacccattattgaacgctttcaagtctacctctggttctatggatgacttgtacaacatgatcaacaccgttaagtctgattgtccagattctactttgttgggtactttcgttgaaaaccacgataatccaagattcgcttcttacaccaacgatattgctttggctaaaaacgttgccgccttcattattttgaacgatggtattccaattatctacgccggtcaagaacaacattatgctggtggtaatgatccagcaaatagagaagctacttggttgtctggttatccaactgattccgagttgtacaaattgattgcttccgctaacgccattagaaactacgctatttctaaggatactggcttcgttacttacaagaattggcctatctacaaggatgataccactattgctatgagaaagggtacagatggttctcaaatcgttaccatcttgtctaacaaaggtgcttctggtgattcctacactttgtctttgtctggtgcaggttatactgctggtcaacaattgactgaagttattggttgtactaccgttaccgttggttctgatggtaatgttcctgttccaatggctggtggtttgccaagagtcttgtatccaacagaaaaattggccggttccaagatctgttcttcttcttga

SEQ ID NO: 105 - protein, 478 aa, Aspergillus oryzae
ATPADWRSQSIYFLLTDRFARTDGSTTATCNTADRKYCGGTWQGIIDKLDYIQGMGFTAIWITPVTAQLPQTTAYGDAYHGYWQQDIYSLNENYGTADDLKALSSALHERGMYLMVDVVANHMGYDGAGSSVDYSVFKPFSSQDYFHPFCLIQNYEDQTQVEDCWLGDNTVSLPDLDTTKDVVKNEWYDWVGSLVSNYSIDGLRIDTVKHVQKDFWPGYNKAAGVYCIGEVLDGDPAYTCPYQNVMDGVLNYPIYYPLLNAFKSTSGSMDDLYNMINTVKSDCPDSTLLGTFVENHDNPRFASYTNDIALAKNVAAFIILNDGIPIIYAGQEQHYAGGNDPANREATWLSGYPTDSELYKLIASANAIRNYAISKDTGFVTYKNWPIYKDDTTIAMRKGTDGSQIVTILSNKGASGDSYTLSLSGAGYTAGQQLTEVIGCTTVTVGSDGNVPVPMAGGLPRVLYPTEKLAGSKICSSS

SEQ ID NO: 106 - DNA, 63 bp, synthetic construct
  misc_feature 1..63: note = Signal peptide from fungal amylase from Aspergillus oryzae
  source 1..63: mol_type = other DNA
atgatggttgcttggtggtctttgttcttgtacggtttacaagttgctgctccagctttggct

SEQ ID NO: 107 - protein, 21 aa, synthetic construct
  REGION 1..21: note = Signal peptide from fungal amylase from Aspergillus oryzae
MMVAWWSLFLYGLQVAAPALA

SEQ ID NO: 108 - protein, 687 aa, Geobacillus stearothermophilus
MSSSASVKGDVIYQIIIDRFYDGDTTNNNPAKSYGLYDPTKSKWKMYWGGDLEGVRQKLPYLKQLGVTTIWLSPVLDNLDTLAGTDNTGYHGYWTRDFKQIEEHFGNWTTFDTLVNDAHQNGIKVIVDFVPNHSTPFKANDSTFAEGGALYNNGTYMGNYFDDATKGYFHHNGDISNWDDRYEAQWKNFTDPAGFSLADLSQENGTIAQYLTDAAVQLVAHGADGLRIDAVKHFNSGFSKSLADKLYQKKDIFLVGEWYGDDPGTANHLEKVRYANNSGVNVLDFDLNTVIRNVFGTFTQTMYDLNNMVNQTGNEYKYKENLITFIDNHDMSRFLSVNSNKANLHQALAFILTSRGTPSIYYGTEQYMAGGNDPYNRGMMPAFDTTTTAFKEVSTLAGLRRNNAAIQYGTTTQRWINNDVYIYERKFFNDVVLVAINRNTQSSYSISGLQTALPNGSYADYLSGLLGGNGISVSNGSVASFTLAPGAVSVWQYSTSASAPQIGSVAPNMGIPGNVVTIDGKGFGTTQGTVTFGGVTATVKSWTSNRIEVYVPNMAAGLTDVKVTAGGVSSNLYSYNILSGTQTSVVFTVKSAPPTNLGDKIYLTGNIPELGNWSTDTSGAVNNAQGPLLAPNYPDWFYVFSVPAGKTIQFKFFIKRADGTIQWENGSNHVATTPTGATGNITVTWQN